European Patent Application EP 4 470 552 A2, published December 4, 2024. Title: HETERODIMERIC FC-FUSED CYTOKINE AND PHARMACEUTICAL COMPOSITION COMPRISING THE SAME. Applicant: AJOU UNIVERSITY INDUSTRY-ACADEMIC COOPERATION FOUNDATION. Application US 18/323,124, filed May 24, 2023. The sequence listing filed with the application follows.

SEQUENCE LISTING (25 sequences)

SEQ ID NO: 1 - protein, 107 aa, synthetic construct
  source 1..107: note = gamma4-EWRVT
GQPREPQVYTLPPSQEEMTENQVSLTCLVKGFYPSDIAVEWESNGQPENNYKTTPPVLDSDGSFFLYSWLTVDKSRWQEGNVFSCSVMHEALHNHYTQKSLSLSLGK

SEQ ID NO: 2 - protein, 107 aa, synthetic construct
  source 1..107: note = gamma4-EWRVT
GQPREPRVYTLPPSQEEMTKNQVSLTCLVKGFYPSDIAVEWESNGQPENNYKTTPPVLVSDGSFTLYSRLTVDKSRWQEGNVFSCSVMHEALHNHYTQKSLSLSLGK

SEQ ID NO: 3 - protein, 107 aa, synthetic construct
  source 1..107: note = gamma4-EWRVTs-s
GQPREPQVCTLPPSQEEMTENQVSLTCLVKGFYPSDIAVEWESNGQPENNYKTTPPVLDSDGSFFLYSWLTVDKSRWQEGNVFSCSVMHEALHNHYTQKSLSLSLGK

SEQ ID NO: 4 - protein, 107 aa, synthetic construct
  source 1..107: note = gamma4-EWRVTs-s
GQPREPRVYTLPPCQEEMTKNQVSLTCLVKGFYPSDIAVEWESNGQPENNYKTTPPVLVSDGSFTLYSRLTVDKSRWQEGNVFSCSVMHEALHNHYTQKSLSLSLGK

SEQ ID NO: 5 - protein, 107 aa, synthetic construct
  source 1..107: note = gamma4-A107
GQPREPQVYTLPPSQEEMTKNQVSLTCLVEGFYPSDIAVEWESNGQPENNYKTTPPVLDSDGSFFLYSWLTVDKSRWQEGNVFSCSVMHEALHNHYTQKSLSLSLGK

SEQ ID NO: 6 - protein, 107 aa, synthetic construct
  source 1..107: note = gamma4-A107
GQPREPQVYTLPPSQENMTKNQVSLTCLVKGFYPSDIAVEWESNGQPENNYKTTPPVLVSDGSFTLYSRLTVDKSRWQEGNVFSCSVMHEALHNHYTQKSLSLSLGK

SEQ ID NO: 7 - protein, 107 aa, synthetic construct
  source 1..107: note = IgG1
GQPREPQVYTLPPSRDELTKNQVSLTCLVKGFYPSDIAVEWESNGQPENNYKTTPPVLDSDGSFFLYSKLTVDKSRWQQGNVFSCSVMHEALHNHYTQKSLSLSPGK

SEQ ID NO: 8 - protein, 107 aa, synthetic construct
  source 1..107: note = gamma1-A107
GQPREPQVYTLPPSRDELTKNQVSLTCLVEGFYPSDIAVEWESNGQPENNYKTTPPVLDSDGSFFLYSWLTVDKSRWQQGNVFSCSVMHEALHNHYTQKSLSLSPGK

SEQ ID NO: 9 - protein, 107 aa, synthetic construct
  source 1..107: note = gamma1-A107
GQPREPQVYTLPPSRDNLTKNQVSLTCLVKGFYPSDIAVEWESNGQPENNYKTTPPVLVSDGSFTLYSKLTVDKSRWQQGNVFSCSVMHEALHNHYTQKSLSLSPGK

SEQ ID NO: 10 - protein, 107 aa, synthetic construct
  source 1..107: note = IgG2
GQPREPQVYTLPPSREEMTKNQVSLTCLVKGFYPSDIAVEWESNGQPENNYKTTPPMLDSDGSFFLYSKLTVDKSRWQQGNVFSCSVMHEALHNHYTQKSLSLSPGK

SEQ ID NO: 11 - protein, 107 aa, synthetic construct
  source 1..107: note = gamma2-A107
GQPREPQVYTLPPSREEMTKNQVSLTCLVEGFYPSDIAVEWESNGQPENNYKTTPPMLDSDGSFFLYSWLTVDKSRWQQGNVFSCSVMHEALHNHYTQKSLSLSPGK

SEQ ID NO: 12 - protein, 107 aa, synthetic construct
  source 1..107: note = gamma2-A107
GQPREPQVYTLPPSRENMTKNQVSLTCLVKGFYPSDIAVEWESNGQPENNYKTTPPMLVSDGSFTLYSKLTVDKSRWQQGNVFSCSVMHEALHNHYTQKSLSLSPGK

SEQ ID NO: 13 - protein, 107 aa, synthetic construct
  source 1..107: note = IgG3
GQPREPQVYTLPPSREEMTKNQVSLTCLVKGFYPSDIAMEWESSGQPENNYKTTPPVLDSDGSFFLYSKLTVDKSRWQQGNIFSCSVMHEALHNHYTQKSLSLSPGK

SEQ ID NO: 14 - protein, 107 aa, synthetic construct
  source 1..107: note = gamma3-A107
GQPREPQVYTLPPSREEMTKNQVSLTCLVEGFYPSDIAMEWESSGQPENNYKTTPPVLDSDGSFFLYSWLTVDKSRWQQGNIFSCSVMHEALHNHYTQKSLSLSPGK

SEQ ID NO: 15 - protein, 107 aa, synthetic construct
  source 1..107: note = gamma3-A107
GQPREPQVYTLPPSRENMTKNQVSLTCLVKGFYPSDIAMEWESSGQPENNYKTTPPVLVSDGSFTLYSKLTVDKSRWQQGNIFSCSVMHEALHNHYTQKSLSLSPGK

SEQ ID NO: 16 - protein, 107 aa, synthetic construct
  source 1..107: note = IgG4
GQPREPQVYTLPPSQEEMTKNQVSLTCLVKGFYPSDIAVEWESNGQPENNYKTTPPVLDSDGSFFLYSRLTVDKSRWQEGNVFSCSVMHEALHNHYTQKSLSLSLGK

SEQ ID NO: 17 - protein, 306 aa, Homo sapiens
IWELKKDVYVVELDWYPDAPGEMVVLTCDTPEEDGITWTLDQSSEVLGSGKTLTIRVKEFGDAGQYTCHKGGEVLSHSLLLLHKKEDGIWSTDILKDQKEPKNKTFLRCEAKNYSGRFTCWWLTTISTDLTFSVKSSRGSSDPQGVTCGAATLSAERVRGDNKEYEYSVECQEDSACPAAEESLPIEVMVDAVHKLKYENYTSSFFIRDIIKPDPPKNLQLKPLKNSRQVEVSWEYPDTWSTPHSYFSLTFCVQVQGKSKREKKDRVFTDKTSATVICRKNASISVRAQDRYYSSSWSEWASVPCS

SEQ ID NO: 18 - protein, 197 aa, Homo sapiens
  source 1..197: note = Mature human IL-12
RNLPVATPDPGMFPCLHHSQNLLRAVSNMLQKARQTLEFYPCTSEEIDHVDITKDKTSTVEACLPLELTKNESCLNSRETSFITNGSCLASRKTSFMMALCLSSIYEDLKMYQVEFKTMNAKLLMDPKRQIFLDQNMLAVIDELMQALNFNSETVPQKSSLEEPDFYKTKIKLCILLHAFRIRAVTIDRVMSYLNAS

SEQ ID NO: 19 - protein, 313 aa, Mus musculus
  source 1..313: note = Mature mouse IL-12
MWELEKDVYVVEVDWTPDAPGETVNLTCDTPEEDDITWTSDQRHGVIGSGKTLTITVKEFLDAGQYTCHKGGETLSHSHLLLHKKENGIWSTEILKNFKNKTFLKCEAPNYSGRFTCSWLVQRNMDLKFNIKSSSSPPDSRAVTCGMASLSAEKVTLDQRDYEKYSVSCQEDVTCPTAEETLPIELALEARQQNKYENYSTSFFIRDIIKPDPPKNLQMKPLKNSQVEVSWEYPDSWSTPHSYFSLKFFVRIQRKKEKMKETKEGCNQKGAFLVEKTSTEVQCKGGNVCVQAQDRYYNSSCSKWACVPCRVRS

SEQ ID NO: 20 - protein, 193 aa, Mus musculus
  source 1..193: note = Mature mouse IL-12
RVIPVSGPARCLSQSRNLLKTTDDMVKTAREKLKHYSCTAEDIDHEDITRDQTSTLKTCLPLELHKNESCLATRETSSTTRGSCLPPQKTSLMMTLCLGSIYEDLKMYQTEFQAINAALQNHNHQQIILDKGMLVAIDELMQSLNHNGETLRQKPPVGEADPYRVKMKLCILLHAFSTRVVTINRVMGYLSSA

SEQ ID NO: 21 - protein, 15 aa, synthetic construct
GGGGSGGGGSGGGGS

SEQ ID NO: 22 - protein, 23 aa, synthetic construct
EPKSSDKTHTCPPCPAPELLGGP

SEQ ID NO: 23 - protein, 19 aa, synthetic construct
ERKSSVECPPCPAPPVAGP

SEQ ID NO: 24 - protein, 23 aa, synthetic construct
EPKSSDTPPPCPRCPAPELLGGP

SEQ ID NO: 25 - protein, 20 aa, synthetic construct
ESKYGPPCPSCPAPEFLGGP